European Patent Specification EP 3 814 347 B1, published May 3, 2023. Title: NAPHTHYRIDINONE COMPOUNDS USEFUL AS T CELL ACTIVATORS. Applicant: BRISTOL-MYERS SQUIBB COMPANY. The sequence listing filed with the application follows.

SEQUENCE LISTING (4 sequences)

SEQ ID NO: 1 - DNA, 2256 bp, Homo sapiens
atggccaaggagaggggcctaataagccccagtgattttgcccagctgcaaaaatacatggaatactccaccaaaaaggtcagtgatgtcctaaagctcttcgaggatggcgagatggctaaatatgtccaaggagatgccattgggtacgagggattccagcaattcctgaaaatctatctcgaagtggataatgttcccagacacctaagcctggcactgtttcaatcctttgagactggtcactgcttaaatgagacaaatgtgacaaaagatgtggtgtgtctcaatgatgtttcctgctacttttcccttctggagggtggtcggccagaagacaagttagaattcaccttcaagctgtacgacacggacagaaatgggatcctggacagctcagaagtggacaaaattatcctacagatgatgcgagtggctgaatacctggattgggatgtgtctgagctgaggccgattcttcaggagatgatgaaagagattgactatgatggcagtggctctgtctctcaagctgagtgggtccgggctggggccaccaccgtgccactgctagtgctgctgggtctggagatgactctgaaggacgacggacagcacatgtggaggcccaagaggttccccagaccagtctactgcaatctgtgcgagtcaagcattggtcttggcaaacagggactgagctgtaacctctgtaagtacactgttcacgaccagtgtgccatgaaagccctgccttgtgaagtcagcacctatgccaagtctcggaaggacattggtgtccaatcacatgtgtgggtgcgaggaggctgtgagtccgggcgctgcgaccgctgtcagaaaaagatccggatctaccacagtctgaccgggctgcattgtgtatggtgccacctagagatccacgatgactgcctgcaagcggtgggccatgagtgtgactgtgggctgctccgggatcacatcctgcctccatcttccatctatcccagtgtcctggcctctggaccggatcgtaaaaatagcaaaacaagccagaagaccatggatgatttaaatttgagcacctctgaggctctgcggattgaccctgttcctaacacccacccacttctcgtctttgtcaatcctaagagtggcgggaagcaggggcagagggtgctctggaagttccagtatatattaaaccctcgacaggtgttcaacctcctaaaggatggtcctgagatagggctccgattattcaaggatgttcctgatagccggattttggtgtgtggtggagacggcacagtaggctggattctagagaccattgacaaagctaacttgccagttttgcctcctgttgctgtgttgcccctgggtactggaaatgatctggctcgatgcctaagatggggaggaggttatgaaggacagaatctggcaaagatcctcaaggatttagagatgagtaaagtggtacatatggatcgatggtctgtggaggtgatacctcaacaaactgaagaaaaaagtgacccagtcccctttcaaatcatcaataactacttctctattggcgtggatgcctctattgctcatcgattccacatcatgcgagagaaatatccggagaagttcaacagcagaatgaagaacaagctatggtacttcgaatttgccacatctgaatccatcttctcaacatgcaaaaagctggaggagtctttgacagttgagatctgtgggaaaccgctggatctgagcaacctgtccctagaaggcatcgcagtgctaaacatccctagcatgcatggtggctccaacctctggggtgataccaggagaccccatggggatatctatgggatcaaccaggccttaggtgctacagctaaagtcatcaccgaccctgatatcctgaaaacctgtgtaccagacctaagtgacaagagactggaagtggttgggctggagggtgcaattgagatgggccaaatctataccaagctcaagaatgctggacgtcggctggccaagtgctctgagatcaccttccacaccacaaaaacccttcccatgcaaattgacggagaaccctggatgcagacgccctgtacaatcaagatcacccacaagaaccagatgcccatgctcatgggcccacccccccgctccaccaatttctttggcttcttgagcggatcctcggagacagtgcggtttcagggacaccaccaccatcaccactga

SEQ ID NO: 2 - protein, 751 aa, Homo sapiens
MAKERGLISPSDFAQLQKYMEYSTKKVSDVLKLFEDGEMAKYVQGDAIGYEGFQQFLKIYLEVDNVPRHLSLALFQSFETGHCLNETNVTKDVVCLNDVSCYFSLLEGGRPEDKLEFTFKLYDTDRNGILDSSEVDKIILQMMRVAEYLDWDVSELRPILQEMMKEIDYDGSGSVSQAEWVRAGATTVPLLVLLGLEMTLKDDGQHMWRPKRFPRPVYCNLCESSIGLGKQGLSCNLCKYTVHDQCAMKALPCEVSTYAKSRKDIGVQSHVWVRGGCESGRCDRCQKKIRIYHSLTGLHCVWCHLEIHDDCLQAVGHECDCGLLRDHILPPSSIYPSVLASGPDRKNSKTSQKTMDDLNLSTSEALRIDPVPNTHPLLVFVNPKSGGKQGQRVLWKFQYILNPRQVFNLLKDGPEIGLRLFKDVPDSRILVCGGDGTVGWILETIDKANLPVLPPVAVLPLGTGNDLARCLRWGGGYEGQNLAKILKDLEMSKVVHMDRWSVEVIPQQTEEKSDPVPFQIINNYFSIGVDASIAHRFHIMREKYPEKFNSRMKNKLWYFEFATSESIFSTCKKLEESLTVEICGKPLDLSNLSLEGIAVLNIPSMHGGSNLWGDTRRPHGDIYGINQALGATAKVITDPDILKTCVPDLSDKRLEVVGLEGAIEMGQIYTKLKNAGRRLAKCSEITFHTTKTLPMQIDGEPWMQTPCTIKITHKNQMPMLMGPPPRSTNFFGFLSGSSETVRFQGHHHHHH

SEQ ID NO: 3 - DNA, 2838 bp, Homo sapiens
atggagccgcgggacggtagccccgaggcccggagcagcgactccgagtcggcttccgcctcgtccagcggctccgagcgcgacgccggtcccgagccggacaaggcgccgcggcgactcaacaagcggcgcttcccggggctgcggctcttcgggcacaggaaagccatcacgaagtcgggcctccagcacctggccccccctccgcccacccctggggccccgtgcagcgagtcagagcggcagatccggagtacagtggactggagcgagtcagcgacatatggggagcacatctggttcgagaccaacgtgtccggggacttctgctacgttggggagcagtactgtgtagccaggatgctgcagaagtcagtgtctcgaagaaagtgcgcagcctgcaagattgtggtgcacacgccctgcatcgagcagctggagaagataaatttccgctgtaagccgtccttccgtgaatcaggctccaggaatgtccgcgagccaacctttgtacggcaccactgggtacacagacgacgccaggacggcaagtgtcggcactgtgggaagggattccagcagaagttcaccttccacagcaaggagattgtggccatcagctgctcgtggtgcaagcaggcataccacagcaaggtgtcctgcttcatgctgcagcagatcgaggagccgtgctcgctgggggtccacgcagccgtggtcatcccgcccacctggatcctccgcgcccggaggccccagaatactctgaaagcaagcaagaagaagaagagggcatccttcaagaggaagtccagcaagaaagggcctgaggagggccgctggagacccttcatcatcaggcccaccccctccccgctcatgaagcccctgctggtgtttgtgaaccccaagagtgggggcaaccagggtgcaaagatcatccagtctttcctctggtatctcaatccccgacaagtcttcgacctgagccagggagggcccaaggaggcgctggagatgtaccgcaaagtgcacaacctgcggatcctggcgtgcgggggcgacggcacggtgggctggatcctctccaccctggaccagctacgcctgaagccgccaccccctgttgccatcctgcccctgggtactggcaacgacttggcccgaaccctcaactggggtgggggctacacagatgagcctgtgtccaagatcctctcccacgtggaggaggggaacgtggtacagctggaccgctgggacctccacgctgagcccaaccccgaggcagggcctgaggaccgagatgaaggcgccaccgaccggttgcccctggatgtcttcaacaactacttcagcctgggctttgacgcccacgtcaccctggagttccacgagtctcgagaggccaacccagagaaattcaacagccgctttcggaataagatgttctacgccgggacagctttctctgacttcctgatgggcagctccaaggacctggccaagcacatccgagtggtgtgtgatggaatggacttgactcccaagatccaggacctgaaaccccagtgtgttgttttcctgaacatccccaggtactgtgcgggcaccatgccctggggccaccctggggagcaccacgactttgagccccagcggcatgacgacggctacctcgaggtcattggcttcaccatgacgtcgttggccgcgctgcaggtgggcggacacggcgagcggctgacgcagtgtcgcgaggtggtgctcaccacatccaaggccatcccggtgcaggtggatggcgagccctgcaagcttgcagcctcacgcatccgcatcgccctgcgcaaccaggccaccatggtgcagaaggccaagcggcggagcgccgcccccctgcacagcgaccagcagccggtgccagagcagttgcgcatccaggtgagtcgcgtcagcatgcacgactatgaggccctgcactacgacaaggagcagctcaaggaggcctctgtgccgctgggcactgtggtggtcccaggagacagtgacctagagctctgccgtgcccacattgagagactccagcaggagcccgatggtgctggagccaagtccccgacatgccagaaactgtcccccaagtggtgcttcctggacgccaccactgccagccgcttctacaggatcgaccgagcccaggagcacctcaactatgtgactgagatcgcacaggatgagatttatatcctggaccctgagctgctgggggcatcggcccggcctgacctcccaacccccacttcccctctccccacctcaccctgctcacccacgccccggtcactgcaaggggatgctgcaccccctcaaggtgaagagctgattgaggctgccaagaggaacgacttctgtaagctccaggagctgcaccgagctgggggcgacctcatgcaccgagacgagcagagtcgcacgctcctgcaccacgcagtcagcactggcagcaaggatgtggtccgctacctgctggaccacgcccccccagagatccttgatgcggtggaggaaaacggggagacctgtttgcaccaagcagcggccctgggccagcgcaccatctgccactacatcgtggaggccggggcctcgctcatgaagacagaccagcagggcgacactccccggcagcgggctgagaaggctcaggacaccgagctggccgcctacctggagaaccggcagcactaccagatgatccagcgggaggaccaggagacggctgtgggatcctcggagacagtgcggtttcagggacaccaccaccatcaccactga

SEQ ID NO: 4 - protein, 945 aa, Homo sapiens
MEPRDGSPEARSSDSESASASSSGSERDAGPEPDKAPRRLNKRRFPGLRLFGHRKAITKSGLQHLAPPPPTPGAPCSESERQIRSTVDWSESATYGEHIWFETNVSGDFCYVGEQYCVARMLQKSVSRRKCAACKIVVHTPCIEQLEKINFRCKPSFRESGSRNVREPTFVRHHWVHRRRQDGKCRHCGKGFQQKFTFHSKEIVAISCSWCKQAYHSKVSCFMLQQIEEPCSLGVHAAVVIPPTWILRARRPQNTLKASKKKKRASFKRKSSKKGPEEGRWRPFIIRPTPSPLMKPLLVFVNPKSGGNQGAKIIQSFLWYLNPRQVFDLSQGGPKEALEMYRKVHNLRILACGGDGTVGWILSTLDQLRLKPPPPVAILPLGTGNDLARTLNWGGGYTDEPVSKILSHVEEGNVVQLDRWDLHAEPNPEAGPEDRDEGATDRLPLDVFNNYFSLGFDAHVTLEFHESREANPEKFNSRFRNKMFYAGTAFSDFLMGSSKDLAKHIRVVCDGMDLTPKIQDLKPQCVVFLNIPRYCAGTMPWGHPGEHHDFEPQRHDDGYLEVIGFTMTSLAALQVGGHGERLTQCREVVLTTSKAIPVQVDGEPCKLAASRIRIALRNQATMVQKAKRRSAAPLHSDQQPVPEQLRIQVSRVSMHDYEALHYDKEQLKEASVPLGTVVVPGDSDLELCRAHIERLQQEPDGAGAKSPTCQKLSPKWCFLDATTASRFYRIDRAQEHLNYVTEIAQDEIYILDPELLGASARPDLPTPTSPLPTSPCSPTPRSLQGDAAPPQGEELIEAAKRNDFCKLQELHRAGGDLMHRDEQSRTLLHHAVSTGSKDVVRYLLDHAPPEILDAVEENGETCLHQAAALGQRTICHYIVEAGASLMKTDQQGDTPRQRAEKAQDTELAAYLENRQHYQMIQREDQETAVGSSETVRFQGHHHHHH